European Patent Specification EP 4 304 631 B1, published October 30, 2024. Title: Treatment of eye diseases with fructosyl-amino acid oxidase. Applicant: Universiteit Gent. The sequence listing filed with the application follows.

SEQUENCE LISTING (4 sequences)

SEQ ID NO: 1 - protein, 325 aa, amino acid
MHHHHHHVNGPGSDEVDEQLLRAELRTATLRAFGGPGAGCISEGRAYDTDAGPVFVKVNRRTQARQMFEGEVASLEALRSTGLVRVPRPMKVIDLPGGGAAFVMEHLKMKSLSSQASKLGEQMADLHLYNQKLREKLKEEENTVGRRGEGAEPQYVDKFGFHTVTCCGFIPQVNEWQDDWPTFFARHRLQAQLDLIEKDYADREARELWSRLQVKIPDLFCGLEIVPALLHGDLWSGNVAEDDVGPIIYDPASFYGHSEFELAIALMFGGFPRSFFTAYHRKIPKAPGFDQRLLLYQLFNYLNHWNHFGREYRSPSLGTMRRLLK

SEQ ID NO: 2 - protein, 308 aa, amino acid
EQLLRAELRTATLRAFGGPGAGCISEGRAYDTDAGPVFVKVNRRTQARQMFEGEVASLEALRSTGLVRVPRPMKVIDLPGGGAAFVMEHLKMKSLSSQASKLGEQMADLHLYNQKLREKLKEEENTVGRRGEGAEPQYVDKFGFHTVTCCGFIPQVNEWQDDWPTFFARHRLQAQLDLIEKDYADREARELWSRLQVKIPDLFCGLEIVPALLHGDLWSGNVAEDDVGPIIYDPASFYGHSEFELAIALMFGGFPRSFFTAYHRKIPKAPGFDQRLLLYQLFNYLNHWNHFGREYRSPSLGTMRRLLK

SEQ ID NO: 3 - DNA, 978 bp, nucleic acid
atgcatcatcatcatcatcatgttaacggtccaggttctgatgaagttgatgaacagttgttgagagctgagttgagaactgctactttgagagcttttggtggtccaggtgctggttgtatttctgagggtagagcttacgatactgacgctggtccagttttcgttaaggttaacagaagaactcaggctagacagatgttcgagggtgaagttgcttctttggaggctttgagatccactggtttggttagagttccaagaccaatgaaggttatcgacttgccaggtggtggtgctgcttttgttatggaacacttgaagatgaagtccttgtcctcccaggcttctaagttgggtgaacaaatggctgacttgcacttgtacaaccagaagttgagagaaaagttgaaagaggaagagaacactgttggtagaagaggtgaaggtgctgagccacaatacgttgacaagttcggtttccacactgttacttgttgtggtttcatcccacaggttaacgagtggcaagatgactggccaactttcttcgctagacacagattgcaagctcagttggacttgatcgagaaggactacgctgacagagaagctagagaattgtggtccagattgcaggttaagatcccagacttgttctgtggtttggagatcgttccagctttgttgcacggtgatttgtggtctggtaacgttgctgaagatgacgttggtccaattatctacgacccagcttctttctacggtcactctgaattcgagttggctatcgctttgatgttcggtggtttcccaagatccttcttcactgcttaccacagaaagatcccaaaggctccaggtttcgaccagagattgttgttgtaccagttgttcaactacttgaaccattggaaccacttcggtagagagtacagatctccatccttgggtactatgagaagattgttgaagtaa

SEQ ID NO: 4 - DNA, 927 bp, nucleic acid
gaacagttgttgagagctgagttgagaactgctactttgagagcttttggtggtccaggtgctggttgtatttctgagggtagagcttacgatactgacgctggtccagttttcgttaaggttaacagaagaactcaggctagacagatgttcgagggtgaagttgcttctttggaggctttgagatccactggtttggttagagttccaagaccaatgaaggttatcgacttgccaggtggtggtgctgcttttgttatggaacacttgaagatgaagtccttgtcctcccaggcttctaagttgggtgaacaaatggctgacttgcacttgtacaaccagaagttgagagaaaagttgaaagaggaagagaacactgttggtagaagaggtgaaggtgctgagccacaatacgttgacaagttcggtttccacactgttacttgttgtggtttcatcccacaggttaacgagtggcaagatgactggccaactttcttcgctagacacagattgcaagctcagttggacttgatcgagaaggactacgctgacagagaagctagagaattgtggtccagattgcaggttaagatcccagacttgttctgtggtttggagatcgttccagctttgttgcacggtgatttgtggtctggtaacgttgctgaagatgacgttggtccaattatctacgacccagcttctttctacggtcactctgaattcgagttggctatcgctttgatgttcggtggtttcccaagatccttcttcactgcttaccacagaaagatcccaaaggctccaggtttcgaccagagattgttgttgtaccagttgttcaactacttgaaccattggaaccacttcggtagagagtacagatctccatccttgggtactatgagaagattgttgaagtaa